European Patent Application EP 4 520 839 A2, published March 12, 2025. Title: Verfahren zur Herstellung von wässerigen Lösungen enthaltend D-Psicose. Applicant: Annikki GmbH. Application EP. The sequence listing filed with the application follows.

SEQUENCE LISTING (20 sequences)

SEQ ID NO: 1 - DNA, 840 bp, Millerozyma farinosa
  source 1..840: mol_type = genomic DNA
atgtctcaagctatctcagcaatcaacgaaagagttggcccattgcccactaaagcaccccaactttcaaaaaacgtattagacctcttttccttgaaaggcaaggtagcatcggtgacaggttcatcgaagggaataggctttgctgtcgcagaagcatacgctcaagcaggggctgatgttgctttgtggtacaattcaagtcctgtcgaggataaggtaaaatacttgaaagagacctacggcgtgaaagtcaaagcctacaagtgtaacgtgggaaacagcgaggaggttgagaaaatagtagaccaaattgcagaggacttcggcacaattgacgtttttgttgctaatgcgggcattgcttggagcgaaggtagatctctcgaggttaagggttacgacgcttggcaaaaaattgtcgactacgacttgagcagtgtatactactgtgctaaggcagtgggtaagatcttccaagaaaagggctccggttcgttaatcctcaccgcatccatgtccggacacattgtgaatgttcctcaaatgcaggcaccatacaatgcggccaaggcggctgtgatccatctaggaaaatctttggctgtcgaatgggctccatttgccagggtcaacaccgtttctcctggctatattgccactgatattggtgaatttgtgctgcccgatgagaagaaaaagtggtggtcattgacacccttgggtagagaaggtcttcctcaagaactcactggtgcatacttgtattttgcttctaacgcatcgacctacactactggggctgacttggtcgtagacggtggctacactgtaccataa

SEQ ID NO: 2 - protein, 279 aa, Millerozyma farinosa
MSQAISAINERVGPLPTKAPQLSKNVLDLFSLKGKVASVTGSSKGIGFAVAEAYAQAGADVALWYNSSPVEDKVKYLKETYGVKVKAYKCNVGNSEEVEKIVDQIAEDFGTIDVFVANAGIAWSEGRSLEVKGYDAWQKIVDYDLSSVYYCAKAVGKIFQEKGSGSLILTASMSGHIVNVPQMQAPYNAAKAAVIHLGKSLAVEWAPFARVNTVSPGYIATDIGEFVLPDEKKKWWSLTPLGREGLPQELTGAYLYFASNASTYTTGADLVVDGGYTVP

SEQ ID NO: 3 - DNA, 785 bp, Gluconobacter frateurii
  source 1..785: mol_type = genomic DNA
atgacacagtctcttcagggcaagatcgtcgccattactggcgcggcttcgggcattggcctcgaatgcgcccgctatctcatcgaagctggcgcggtggtctatcttctggaccgtgacgccaaaactctcgaagacaaaacggcagaactcggcagccaggcccatgcgatcatcgtcgatctcttcgactacaaaaccgtagatgctgcggtcgcgcagatcgttgaggagcagggccggatcgatgttttccacgccaacgccggcgcgtatgtgggcggcaatgtctgggaaggggatcccgatagctgggatgcgatgctgcacctgaacatcaatgcagctttccgctcggtccgtgccgtgctgccgcagatgatgaagcaggaaagtggcgatatcgtcatgaccagctcgatcgcgggcatgatccccatcatggccgagccgatctacacggcctcgaaacatgccgtgcaggcattcgtacatacggtgcgccgacaggtcgcgaagtatggaattcgtgtgggtgcaatccagcctggtcctgtagtcacgcctttgctgaaagactgggatcaggcccgtcttgaagccaacatcaaagcgggtgccctgatggaagccaaggaagtcgccgaagccctgatcttcatcctgacacgttcaaagggtgtcatggtgcgggatctggtcgttctgccacataacttcgacgcctaagcttaagcggccgcactcgagcaccaccaccaccaccactgagatccggctgctaa

SEQ ID NO: 4 - protein, 242 aa, Gluconobacter frateurii
MTQSLQGKIVAITGAASGIGLECARYLIEAGAVVYLLDRDAKTLEDKTAELGSQAHAIIVDLFDYKTVDAAVAQIVEEQGRIDVFHANAGAYVGGNVWEGDPDSWDAMLHLNINAAFRSVRAVLPQMMKQESGDIVMTSSIAGMIPIMAEPIYTASKHAVQAFVHTVRRQVAKYGIRVGAIQPGPVVTPLLKDWDQARLEANIKAGALMEAKEVAEALIFILTRSKGVMVRDLVVLPHNFDA

SEQ ID NO: 5 - DNA, 1062 bp, Galactocandida mastotermitis
  source 1..1062: mol_type = genomic DNA
atgagcacaccggaaaatctgagctttgtgctgcagaaaccgtttgatgtgaaatttgaagatcgtccgattccgaaactgagcgatccgtatagcgttaaaattcaggtgaaaaaaaccggcatttgcggtagtgatgttcactatttcacccatggtgcaattggtgattttgttgttaaagcaccgatggttctgggtcatgaaagcagcggtgttgttctggaagttggtagcgaagttaaaagcctgaaagttggtgatcgtgttgcaatggaaccgggtgttccgagccgtcatagtgatgagtataaaagcggtcgttataatctgtgtccgcacatggcatttgcagcaacccctccgtatgatggcaccctgtgtaaatactatattctgccggaagatttctgcgttaaactgccggaacatgttagcctggaagaaggtgcactggttgaaccgctgagcgttgcagttcatagcagcaaactgggtaacattaaaccgggtagccatgttgcaatttatggtgcaggtccggttggtctgctggttgcagcagttgcaagcgcatttggtgcagaaagcgttaccattattgatctggttgaaagccgtctgaatctggcaaaagaactgggtgcaaccgcaaccgttcaggttgattttaaagataccccgaaagaaagcgcagcaaaagttgttgcagcaaataatggcattgcaccggatgttgttattgatgcaagcggtgcagaagcaagcattaattcagccattaatgcaattcgtccgggtggcacctatgttcaggtgggtatgggtaaaccggatgtgagctttccgattgcaaccctgattggtaaagaactgaccgttaaaggtagctttcgttatggttatggtgattatccgctggcagttagcctgctggcaagcggtaaagttaatgtgaaaaaactgatcacccatgaagtgaaattcgaggatgcagcagaagcatttcagctggttcgtgatggtaaagccattaaatgtattatcaacggtccggaataa

SEQ ID NO: 6 - protein, 353 aa, Galactocandida mastotermitis
MSTPENLSFVLQKPFDVKFEDRPIPKLSDPYSVKIQVKKTGICGSDVHYFTHGAIGDFVVKAPMVLGHESSGVVLEVGSEVKSLKVGDRVAMEPGVPSRHSDEYKSGRYNLCPHMAFAATPPYDGTLCKYYILPEDFCVKLPEHVSLEEGALVEPLSVAVHSSKLGNIKPGSHVAIYGAGPVGLLVAAVASAFGAESVTIIDLVESRLNLAKELGATATVQVDFKDTPKESAAKVVAANNGIAPDVVIDASGAEASINSAINAIRPGGTYVQVGMGKPDVSFPIATLIGKELTVKGSFRYGYGDYPLAVSLLASGKVNVKKLITHEVKFEDAAEAFQLVRDGKAIKCIINGPE

SEQ ID NO: 7 - DNA, 1062 bp, Priestia megaterium
  source 1..1062: mol_type = genomic DNA
atgaataacaacctgccgaaaaccatgaaagcagcagttatgcatggcacccgtgaaattagcattgaaaccctgccgattccgcagattgatgaaaatgaagttctgatcaaagttatggccgttggtatttgtggtagcgatctgcactattacacccagggtcgtattggtaaatacaaagtggaaaaaccgtttatcctgggtcatgaatgtagcggtgaagttgttgcaattggtagcgcagttgaacgttttcgtgttggtgatcgtgttgccgttgaaccgggtgttacctgtggtcattgtgaagcatgtaaagagggtcgttataatctgtgtccggatgttcagtttctggcaacccctccggttgatggtgcatttgttcagtatatcaaaatgcgccaggatttcgtttttctgattccgaatagcctgagctatgaagatgcagcactgattgaaccgtttagcgtgggtattcatgcagcaacccgtaccaaactgcagcctggtagcaccattgcaattatgggtatgggtccggttggtctgatggcagttgcagcagcaaaagcatttggtgcaagcaccattattgcaaccgatctggaaccgctgcgtctggaagcagccaaacgtatgggtgcaacccatgttattaacattcgtgaacaggatccgctgaacgagattaaaaacattaccgaaaatgtgggtgttgatgttgcatgggaaaccgcaggtaatccgaaagcactgcagagcagcctgagcagcattcgtcgtggtggtaaactggcaattgttggtctgccgagccagagcgatattccgctggatgttccgtttattgccgataatgaaatcgatatctatggcatctttcgctatgcaaacacctatccgaaaggcatcaaatttctgaccagcggtgcaattgataccaaaaatctggttaccgatcgttatccgctggcaggtacacgtgaagcaatggaacgtgcactgaatttcaaaaacgaatgcctgaaaatcatcgtgtatccgaacgaataa

SEQ ID NO: 8 - protein, 353 aa, Priestia megaterium
MNNNLPKTMKAAVMHGTREISIETLPIPQIDENEVLIKVMAVGICGSDLHYYTQGRIGKYKVEKPFILGHECSGEVVAIGSAVERFRVGDRVAVEPGVTCGHCEACKEGRYNLCPDVQFLATPPVDGAFVQYIKMRQDFVFLIPNSLSYEDAALIEPFSVGIHAATRTKLQPGSTIAIMGMGPVGLMAVAAAKAFGASTIIATDLEPLRLEAAKRMGATHVINIREQDPLNEIKNITENVGVDVAWETAGNPKALQSSLSSIRRGGKLAIVGLPSQSDIPLDVPFIADNEIDIYGIFRYANTYPKGIKFLTSGAIDTKNLVTDRYPLAGTREAMERALNFKNECLKIIVYPNE

SEQ ID NO: 9 - DNA, 729 bp, Kozakia baliensis
  source 1..729: mol_type = genomic DNA
atgacctctcctctccagggtaagatagccgccatcacgggcggggcttcgggcatcggcctcgaatgtgtccgccagatcgccgcaagtggtgccacggtttatattctcgaccgcgaccatcaggcgctcgacaaggcgcgcgaagaattgggcgagcgcgttcataccatcgaggtcgatctcttccgttacgaaacggtcgatcgcgccatcgaaaccatcgtgtccgaacaaggacgcatcgacattctccatgtcaatgcgggcgcgtatatcggcggcaatgtctgggaaggcgatcccgataaatgggacaagatgctgaatctcaacatcaacgccgccttccgttccgcccgcgccgtcatgcccgccatgatgaagcagaaaagcggcgatatcatcatgacaagctcgatcgcaggcatcgtcccgatcccggcggagccgatctacacggcttccaaacatgcggtgcaagccttcgctcacaccatacgccgccagttggccccgttcggcatccgcgtcggcgccatccagcccggcccggtcgtcacgcccttgctcaatgattgggaccccgagcgccttaaagccaatatcgaggctggcgccatgatgcagccttctgacgtcgccgaagccgtggttttcatgctgtcccgccgcaagggaacggtaatccgcgacttggttctgttaccccattctttcgacgtctaa

SEQ ID NO: 10 - protein, 242 aa, Kozakia baliensis
MTSPLQGKIAAITGGASGIGLECVRQIAASGATVYILDRDHQALDKAREELGERVHTIEVDLFRYETVDRAIETIVSEQGRIDILHVNAGAYIGGNVWEGDPDKWDKMLNLNINAAFRSARAVMPAMMKQKSGDIIMTSSIAGIVPIPAEPIYTASKHAVQAFAHTIRRQLAPFGIRVGAIQPGPVVTPLLNDWDPERLKANIEAGAMMQPSDVAEAVVFMLSRRKGTVIRDLVLLPHSFDV

SEQ ID NO: 11 - DNA, 729 bp, Providencia heimbachae
  source 1..729: mol_type = genomic DNA
atggctatatctctcgaaaacaacgtagctgcaattacaggtgccgcttcaggtatcggtctcgaatgtgcacgcacactgatcaaagcaggcgctaaagttgtcctcattgaccgagcagaagatagactaaatcaattggtcgcagaattaggtgaaaatgcaattccattagttatcgatttaatgaaaccagaacaagtcgatggcatgttagcgcgtattatcgaaaaggcaggcagattagatatctttcatgctaatgctggagcttacattggtgggcccgtagccgaaggcgatcccgatgtttgggataaagtcctaaatttaaatgttaatgccgcattccgctgtgttcgcgcagttctaccacactttatcgcacaaaagtcaggcgatattctattcaccagctctatcgctggtatggttcccgtaatttgggagcctatttacacggcatcaaaatttgcggttcaagcattcgttcattctactcgccgtcaggtttctgaacacggtgtccgtgttggtgctgtattacctggtcctgttgttactgcgttattagatgattggccaaaagaaaaacttgaagaagctttagctaacggtagtttaatgcaacccattgaagttgctgaggctgttctattcatgctgacgcgtccaagaaatattacaattcgcgatttagttattttacccaatagtgttgacctctaa

SEQ ID NO: 12 - protein, 242 aa, Providencia heimbachae
MAISLENNVAAITGAASGIGLECARTLIKAGAKVVLIDRAEDRLNQLVAELGENAIPLVIDLMKPEQVDGMLARIIEKAGRLDIFHANAGAYIGGPVAEGDPDVWDKVLNLNVNAAFRCVRAVLPHFIAQKSGDILFTSSIAGMVPVIWEPIYTASKFAVQAFVHSTRRQVSEHGVRVGAVLPGPVVTALLDDWPKEKLEEALANGSLMQPIEVAEAVLFMLTRPRNITIRDLVILPNSVDL

SEQ ID NO: 13 - DNA, 1374 bp, unidentified
  source 1..1374: mol_type = genomic DNA
atgagcaaaattgttatcgtgggtgcaaatcatgcaggcaccgcagcaattaataccattctggataattatggcagcgaaaatgaagtggttgtgtttgatcagaatagcaacattagctttctgggttgtggtatggcactgtggattggtaaacaaattagcggtccgcagggtctgttttatgcagataaagaaagcctggaagcaaaaggtgccaaaatctatatggaaagtccggttaccgccattgattatgatgcaaaacgtgttaccgcactggttaatggtcaagaacatgttgaaagctacgagaaactgattctggcaaccggtagcaccccgattctgcctccgattaaaggtgcagccattaaagaaggtagtcgcgattttgaagcaaccctgaaaaatctgcagttcgtgaaactgtatcagaatgccgaagatgtgattaacaaactgcaggataaaagccagaatctgaatcgtattgcagttgttggtgcaggttatattggtgttgaactggcagaagcatttaaacgtctgggtaaagaagtgattctgattgacgttgttgatacctgtctggcaggttattatgatcaggatctgagcgaaatgatgcgtcagaatctggaagatcatggtatcgaactggcatttggtgaaaccgttaaagcaattgaaggtgatggtaaagtggaacgtattgttaccgataaagcaagccatgatgtggatatggttattctggcagttggttttcgtccgaatacagcactgggtaatgcaaaactgaaaacctttcgtaatggtgcctttctggtggataaaaaacaagaaaccagcatcccggatgtttatgcaattggtgattgtgcaaccgtgtatgataatgccattaacgacaccaactatattgcactggcaagcaatgcactgcgtagcggtattgttgcaggtcataatgcagccggtcataaactggaaagtctgggtgttcagggtagcaatggtatttcaatttttggcctgaatatggttagcaccggtctgacccaagaaaaagccaaacgttttggttataatccggaagttaccgcctttaccgattttcagaaagccagctttatcgagcatgataactatccggttacgctgaaaattgtgtatgacaaagatagccgtctggttctgggtgcacagatggccagcaaagaagatatgagcatgggtattcacatgtttagcctggccattcaagagaaagttaccattgaacgtctggccctgctggattatttctttctgccgcattttaatcagccgtacaactatatgaccaaagcagcactgaaagccaaataa

SEQ ID NO: 14 - protein, 457 aa, unidentified
MSKIVIVGANHAGTAAINTILDNYGSENEVVVFDQNSNISFLGCGMALWIGKQISGPQGLFYADKESLEAKGAKIYMESPVTAIDYDAKRVTALVNGQEHVESYEKLILATGSTPILPPIKGAAIKEGSRDFEATLKNLQFVKLYQNAEDVINKLQDKSQNLNRIAVVGAGYIGVELAEAFKRLGKEVILIDVVDTCLAGYYDQDLSEMMRQNLEDHGIELAFGETVKAIEGDGKVERIVTDKASHDVDMVILAVGFRPNTALGNAKLKTFRNGAFLVDKKQETSIPDVYAIGDCATVYDNAINDTNYIALASNALRSGIVAGHNAAGHKLESLGVQGSNGISIFGLNMVSTGLTQEKAKRFGYNPEVTAFTDFQKASFIEHDNYPVTLKIVYDKDSRLVLGAQMASKEDMSMGIHMFSLAIQEKVTIERLALLDYFFLPHFNQPYNYMTKAALKAK

SEQ ID NO: 15 - DNA, 1356 bp, Carnobacterium divergens
  source 1..1356: mol_type = genomic DNA
atgaaagtagtagtagtaggctgtacacatgcaggaacagcggcagttaagacgattttaaatgaacatccagatgcatcagtatcagtatatgagcgtaatgacaatgtctcatttctatcttgtgggattgcgttgtatgttggtggagttgtgaaagatcctgcaggtttgttttattcaagtccagaagaacttgcatcaatgggcgcgaaaattaacatggaacacaatgtgaaaaatatagataatgagaataaggtcgtagtaattgagaatttaaaaacaggcgaaacatttgaagaaagctatgataagttggtaatgacaactggatcatggccaattattcctccaattgatggaatcaatagtgaaaatattcttttgtgtaaaaactataaccaagcaaatgaaattattaaagaatcaaaaaatgctaaaaagattgtcattgttggtggtggctatattggaattgaattagttgaggcatttgcagaatctggcaagcaagtgacgctagttgatggattagatcgtattttaaacaaatatttagatgctgaattcacttctgttttagagcatgatttacaagaaagaggcgttacgctagctttaaaccaaaccgtcgagaaatttgttgccaatgaatcaggtgctgtgacagctgtgaaaacaccagttggagaatatgaggctgatttagttattttatgtgttggatttaaaccaaatactgatttgttgaaggataaagtagagatgttgccaaatggtgccatcgtagtggatgaatatatgagaacaagcgatgaagcgatttttgctgctggcgatagttgcgcggttcattataatccaactggaggctctgcgtatattccgttagctacaaatgcagttagaatgggagctttagttgggaaaaatattgtttctccaacagttaaatatcgtggcacgcaagcaacttctggtttatatttatttggttttaatataggttcaaccggattgactgaaaatagcgctcctcattttggcgtagaggttcgttcagtagttgtagaagataattatcgtccagagtttatgccgacaacagagaaagtaacgatgaaattagtttatgaagtaggaacgaatcggattgttggaggtcaaatcatgtcaaaatatgatgtgacacaatctgccaatacgttatctttatgtgttcaaaataaaatgacgattgaggatttggcttatgtagatttcttcttccaacctcactttgatcgtccttggaactatttaaatattttagcgcaagcagctgttgagcaagagcgtaaactagcaaaataa

SEQ ID NO: 16 - protein, 451 aa, Carnobacterium divergens
MKVVVVGCTHAGTAAVKTILNEHPDASVSVYERNDNVSFLSCGIALYVGGVVKDPAGLFYSSPEELASMGAKINMEHNVKNIDNENKVVVIENLKTGETFEESYDKLVMTTGSWPIIPPIDGINSENILLCKNYNQANEIIKESKNAKKIVIVGGGYIGIELVEAFAESGKQVTLVDGLDRILNKYLDAEFTSVLEHDLQERGVTLALNQTVEKFVANESGAVTAVKTPVGEYEADLVILCVGFKPNTDLLKDKVEMLPNGAIVVDEYMRTSDEAIFAAGDSCAVHYNPTGGSAYIPLATNAVRMGALVGKNIVSPTVKYRGTQATSGLYLFGFNIGSTGLTENSAPHFGVEVRSVVVEDNYRPEFMPTTEKVTMKLVYEVGTNRIVGGQIMSKYDVTQSANTLSLCVQNKMTIEDLAYVDFFFQPHFDRPWNYLNILAQAAVEQERKLAK

SEQ ID NO: 17 - DNA, 1014 bp, Geobacillus stearothermophilus
  source 1..1014: mol_type = genomic DNA
atgaaagctgcagttgtggaacaatttaaaaagccgttacaagtgaaagaagtggaaaaacctaagatctcatacggggaagtattagtgcgcatcaaagcgtgtggggtatgccatacagacttgcatgccgcacatggcgactggcctgtaaagcctaaactgcctctcattcctggccatgaaggcgtcggtgtaattgaagaagtaggtcctggggtaacacatttaaaagttggagatcgcgtaggtatcccttggctttattcggcgtgcggtcattgtgactattgcttaagcggacaagaaacattatgcgaacgtcaacaaaacgctggctattccgtcgatggtggttatgctgaatattgccgtgctgcagccgattatgtcgtaaaaattcctgataacttatcgtttgaagaagccgctccaatcttttgcgctggtgtaacaacatataaagcgctcaaagtaacaggcgcaaaaccaggtgaatgggtagccatttacggtatcggcgggcttggacatgtcgcagtccaatacgcaaaggcgatggggttaaacgtcgttgctgtcgatttaggtgatgaaaaacttgagcttgctaaacaacttggtgcagatcttgtcgtcaatccgaaacatgatgatgcagcacaatggataaaagaaaaagtgggcggtgtgcatgcgactgtcgtcacagctgtttcaaaagccgcgttcgaatcagcctacaaatccattcgtcgcggtggtgcttgcgtactcgtcggattaccgccggaagaaatacctattccaattttcgatacagtattaaatggagtaaaaattattggttctatcgttggtacgcgcaaagacttacaagaggcacttcaatttgcagcagaaggaaaagtaaaaacaattgtcgaagtgcaaccgcttgaaaacattaacgacgtattcgatcgtatgttaaaagggcaaattaacggccgcgtcgtgttaaaagtagattaa

SEQ ID NO: 18 - protein, 337 aa, Geobacillus stearothermophilus
MKAAVVEQFKKPLQVKEVEKPKISYGEVLVRIKACGVCHTDLHAAHGDWPVKPKLPLIPGHEGVGVIEEVGPGVTHLKVGDRVGIPWLYSACGHCDYCLSGQETLCERQQNAGYSVDGGYAEYCRAAADYVVKIPDNLSFEEAAPIFCAGVTTYKALKVTGAKPGEWVAIYGIGGLGHVAVQYAKAMGLNVVAVDLGDEKLELAKQLGADLVVNPKHDDAAQWIKEKVGGVHATVVTAVSKAAFESAYKSIRRGGACVLVGLPPEEIPIPIFDTVLNGVKIIGSIVGTRKDLQEALQFAAEGKVKTIVEVQPLENINDVFDRMLKGQINGRVVLKVD

SEQ ID NO: 19 - DNA, 786 bp, Priestia megaterium
  source 1..786: mol_type = genomic DNA
atgtatacagatttaaaagataaagtagttgtaattacaggtggatcaacaggtttaggacgcgcaatggctgttcgtttcggtcaagaagaagcaaaagttgttattaactattacaacaatgaagaagaagctttagatgcgaaaaaagaagtagaagaagcaggcggacaagcaatcatcgttcaaggcgacgtaacaaaagaagaagatgttgtaaaccttgttcaaacagctattaaagaattcggtacattagacgttatgattaataacgctggtgttgaaaacccagttccttctcatgagttatctttagacaactggaataaagttattgatacaaacttaacaggtgcattcttaggaagccgtgaagcaatcaaatattttgttgaaaacgacattaaaggaaacgttattaacatgtctagtgttcatgaaatgattccttggccattatttgttcattacgcagcaagtaaaggcggtatgaaactaatgacggaaacattggctcttgaatatgcgccaaaaggtatccgcgtaaataacattggaccaggtgcgatgaacacaccaattaacgcagagaaatttgcagatcctgtacaacgtgcagacgtagaaagcatgattccaatgggttacatcggtaaaccagaagaagtagcagcagttgcagcattcttagcatcatcacaagcaagctatgtaacaggtattacattatttgctgatggtggtatgacgaaatacccttctttccaagcaggaagaggctaa

SEQ ID NO: 20 - protein, 261 aa, Priestia megaterium
MYTDLKDKVVVITGGSTGLGRAMAVRFGQEEAKVVINYYNNEEEALDAKKEVEEAGGQAIIVQGDVTKEEDVVNLVQTAIKEFGTLDVMINNAGVENPVPSHELSLDNWNKVIDTNLTGAFLGSREAIKYFVENDIKGNVINMSSVHEMIPWPLFVHYAASKGGMKLMTETLALEYAPKGIRVNNIGPGAMNTPINAEKFADPVQRADVESMIPMGYIGKPEEVAAVAAFLASSQASYVTGITLFADGGMTKYPSFQAGRG